European Patent Specification EP 2 989 889 B1, published May 24, 2023. Title: Generation of haploid plants. Applicant: IPK Gatersleben. The sequence listing filed with the application follows.

SEQUENCE LISTING (48 sequences)

SEQ ID NO: 1 - protein, 29 aa, plant
  misc_feature (1)..(2): Xaa can be any naturally occurring amino acid
  misc_feature (5)..(7): Xaa can be any naturally occurring amino acid
  misc_feature (10)..(11): Xaa can be any naturally occurring amino acid
  misc_feature (13)..(18): Xaa can be any naturally occurring amino acid
  misc_feature (20)..(24): Xaa can be any naturally occurring amino acid
  misc_feature (29)..(29): Xaa can be any naturally occurring amino acid
XXALXXXQEXXEXXXXXXFXXXXXCAIHX

SEQ ID NO: 2 - DNA, 20 bp, artificial sequence
  artificial DNA
  misc_feature: artificial
aggcagggtctcaattcctt

SEQ ID NO: 3 - DNA, 20 bp, artificial sequence
  artificial DNA
gtcccatcatccatcgtctt

SEQ ID NO: 4 - DNA, 20 bp, artificial sequence
  artificial DNA
cccacttccttgttgtggac

SEQ ID NO: 5 - DNA, 23 bp, artificial sequence
  artificial DNA
ggcgataaatgtatcttgcattc

SEQ ID NO: 6 - DNA, 20 bp, artificial sequence
  artificial DNA
tggtagcaaccagagctacg

SEQ ID NO: 7 - DNA, 20 bp, artificial sequence
  artificial DNA
actggcatgtttccttctgc

SEQ ID NO: 8 - DNA, 20 bp, artificial sequence
  artificial DNA
cggacggagggagtatttct

SEQ ID NO: 9 - DNA, 20 bp, artifical sequence
ggacatgcccaaagaaagtg

SEQ ID NO: 10 - DNA, 21 bp, artificial sequence
  artificial DNA
gccagcgagtactcctacaag

SEQ ID NO: 11 - DNA, 21 bp, artificial sequence
  artificial DNA
ttgagttaccagccaccactc

SEQ ID NO: 12 - DNA, 20 bp, artificial sequence
  artificial DNA
gtcatgcactgtgtcttgca

SEQ ID NO: 13 - DNA, 22 bp, artificial sequence
  artificial DNA
tgctaagatcggataactgtgg

SEQ ID NO: 14 - DNA, 21 bp, artificial sequence
  artificial DNA
tgctcctgaacaaactgaacc

SEQ ID NO: 15 - DNA, 19 bp, artificial sequence
  artificial DNA
gtggccgtcagtacaatcg

SEQ ID NO: 16 - DNA, 26 bp, artificial sequence
  artificial DNA
ggatccatgagagttaaacacactgc

SEQ ID NO: 17 - DNA, 26 bp, artificial sequence
  artificial DNA
ggatcctgttcagttaccatcccctc

SEQ ID NO: 18 - DNA, 28 bp, artificial sequence
  artificial DNA
atggatccatgagagttaaacacactgc

SEQ ID NO: 19 - DNA, 30 bp, artificial sequence
  artificial DNA
ctctgcagcctcttgaagggccataaaagc

SEQ ID NO: 20 - DNA, 30 bp, artificial sequence
  artificial DNA
ctctgcagcctcttgaagggccataatagc

SEQ ID NO: 21 - DNA, 24 bp, artificial sequence
  artificial DNA
caatgatagctgcaccaccaactg

SEQ ID NO: 22 - DNA, 23 bp, artificial sequence
  artificial DNA
ctagctgcccttccacctctcca

SEQ ID NO: 23 - DNA, 22 bp, artificial sequence
  artificial DNA
agtcggtcaattttctcatccc

SEQ ID NO: 24 - DNA, 21 bp, artificial sequence
  artificial DNA
ctctgtagcctcttgaactgc

SEQ ID NO: 25 - DNA, 20 bp, artificial sequence
  artificial DNA
gccattgtcgaacaagaagg

SEQ ID NO: 26 - DNA, 20 bp, artificial sequence
  artificial DNA
taacacggtgcgaatgaatg

SEQ ID NO: 27 - DNA, 26 bp, artificial sequence
  artificial DNA
gacagctgaagcatttgttgctcttc

SEQ ID NO: 28 - DNA, 26 bp, artificial sequence
  artificial DNA
gacagctgaagctattgttgctcttc

SEQ ID NO: 29 - DNA, 21 bp, artificial sequence
  artificial DNA
caacgattgatttggggaggg

SEQ ID NO: 30 - DNA, 27 bp, artificial sequence
  artificial DNA
ggtgcgatttctccagcagtaaaaatc

SEQ ID NO: 31 - DNA, 26 bp, artificial sequence
  artificial DNA
ctgagaagatgaagcaccggcgatat

SEQ ID NO: 32 - DNA, 25 bp, artificial sequence
  artificial DNA
aacttttgccatcctcgtttctgtt

SEQ ID NO: 33 - DNA, 420 bp, Hordeum vulgare
atggctcgcacgaagaaaacggtggcggcgaaggagaagcgccccccttgctccaagtcggagccgcagtcgcagccgaagaagaaggagaagcgggcgtaccggttccggccgggcacggtggcgctgcgggagatccggaagtaccgcaagtccaccaatatgctcatcccctttgcgcccttcgtccgcctggtcagggacatcgccgacaacttgacgccattgtcgaacaagaaggagagcaagccgacgccatggactcctctcgcgctcctctcgttgcaagagtctgcagagtatcacttggtcgatctatttggaaaggcaaatctgtgtgccattcattcgcaccgtgttaccatcatgctaaaggacatgcagcttgcgaggcgtatcgggacgagaagcctttggtga

SEQ ID NO: 34 - protein, 139 aa, Hordeum vulgare
MARTKKTVAAKEKRPPCSKSEPQSQPKKKEKRAYRFRPGTVALREIRKYRKSTNMLIPFAPFVRLVRDIADNLTPLSNKKESKPTPWTPLALLSLQESAEYHLVDLFGKANLCAIHSHRVTIMLKDMQLARRIGTRSLW

SEQ ID NO: 35 - DNA, 420 bp, Hordeum vulgare (Tilling Line 4528 Mutant)
atggctcgcacgaagaaaacggtggcggcgaaggagaagcgccccccttgctccaagtcggagccgcagtcgcagccgaagaagaaggagaagcgggcgtaccggttccggccgggcacggtggcgctgcgggagatccggaagtaccgcaagtccaccaatatgctcatcccctttgcgcccttcgtccgcctggtcagggacatcgccgacaacttgacgccattgtcgaacaagaaggagagcaagccgacgccatggactcctctcgcgttcctctcgttgcaagagtctgcagagtatcacttggtcgatctatttggaaaggcaaatctgtgtgccattcattcgcaccgtgttaccatcatgctaaaggacatgcagcttgcgaggcgtatcgggacgagaagcctttggtga

SEQ ID NO: 36 - protein, 139 aa, Hordeum vulgare (Tilling Line 4528 Mutant)
MARTKKTVAAKEKRPPCSKSEPQSQPKKKEKRAYRFRPGTVALREIRKYRKSTNMLIPFAPFVRLVRDIADNLTPLSNKKESKPTPWTPLAFLSLQESAEYHLVDLFGKANLCAIHSHRVTIMLKDMQLARRIGTRSLW

SEQ ID NO: 37 - DNA, 537 bp, Arabidopsis thaliana
atggcgagaaccaagcatcgcgttaccaggtcacaacctcggaatcaaactgatgccgccggtgcttcatcttctcaggcggcaggtccaactacgaccccgacaaggagaggcggtgaaggtggagataatactcaacaaacaaatcctacaacttcaccagctactggtacaaggagaggggctaagagatccagacaggctatgccacgaggctcacagaagaagtcttatcgatacaggccaggaaccgttgctctaaaagagattcgccatttccagaagcagacaaaccttcttattccggctgccagtttcataagagaagtgagaagtataacccatatgttggcccctccccaaatcaatcgttggacagctgaagctcttgttgctcttcaagaggcggcagaagattacttggttggtttgttctcagattcaatgctctgtgctatccatgcaagacgtgttactctaatgagaaaagactttgaacttgcacgccggcttggaggaaaaggcagaccatggtga

SEQ ID NO: 38 - protein, 178 aa, Arabidopsis thaliana
MARTKHRVTRSQPRNQTDAAGASSSQAAGPTTTPTRRGGEGGDNTQQTNPTTSPATGTRRGAKRSRQAMPRGSQKKSYRYRPGTVALKEIRHFQKQTNLLIPAASFIREVRSITHMLAPPQINRWTAEALVALQEAAEDYLVGLFSDSMLCAIHARRVTLMRKDFELARRLGGKGRPW

SEQ ID NO: 39 - DNA, 537 bp, Arabidopsis thaliana
atggcgagaaccaagcatcgcgttaccaggtcacaacctcggaatcaaactgatgccgccggtgcttcatcttctcaggcggcaggtccaactacgaccccgacaaggagaggcggtgaaggtggagataatactcaacaaacaaatcctacaacttcaccagctactggtacaaggagaggggctaagagatccagacaggctatgccacgaggctcacagaagaagtcttatcgatacaggccaggaaccgttgctctaaaagagattcgccatttccagaagcagacaaaccttcttattccggctgccagtttcataagagaagtgagaagtataacccatatgttggcccctccccaaatcaatcgttggacagctgaagctattgttgctcttcaagaggcggcagaagattacttggttggtttgttctcagattcaatgctctgtgctatccatgcaagacgtgttactctaatgagaaaagactttgaacttgcacgccggcttggaggaaaaggcagaccatggtga

SEQ ID NO: 40 - protein, 178 aa, Arabidopsis thaliana
MARTKHRVTRSQPRNQTDAAGASSSQAAGPTTTPTRRGGEGGDNTQQTNPTTSPATGTRRGAKRSRQAMPRGSQKKSYRYRPGTVALKEIRHFQKQTNLLIPAASFIREVRSITHMLAPPQINRWTAEAIVALQEAAEDYLVGLFSDSMLCAIHARRVTLMRKDFELARRLGGKGRPW

SEQ ID NO: 41 - DNA, 537 bp, Arabidopsis thaliana
atggcgagaaccaagcatcgcgttaccaggtcacaacctcggaatcaaactgatgccgccggtgcttcatcttctcaggcggcaggtccaactacgaccccgacaaggagaggcggtgaaggtggagataatactcaacaaacaaatcctacaacttcaccagctactggtacaaggagaggggctaagagatccagacaggctatgccacgaggctcacagaagaagtcttatcgatacaggccaggaaccgttgctctaaaagagattcgccatttccagaagcagacaaaccttcttattccggctgccagtttcataagagaagtgagaagtataacccatatgttggcccctccccaaatcaatcgttggacagctgaagcatttgttgctcttcaagaggcggcagaagattacttggttggtttgttctcagattcaatgctctgtgctatccatgcaagacgtgttactctaatgagaaaagactttgaacttgcacgccggcttggaggaaaaggcagaccatggtga

SEQ ID NO: 42 - protein, 178 aa, Arabidopsis thaliana
MARTKHRVTRSQPRNQTDAAGASSSQAAGPTTTPTRRGGEGGDNTQQTNPTTSPATGTRRGAKRSRQAMPRGSQKKSYRYRPGTVALKEIRHFQKQTNLLIPAASFIREVRSITHMLAPPQINRWTAEAFVALQEAAEDYLVGLFSDSMLCAIHARRVTLMRKDFELARRLGGKGRPW

SEQ ID NO: 43 - DNA, 465 bp, Beta vulgaris
atgagagttaaacacactgctgccaggaaatcaaccaccaatggtcctcgttcaaaggctcagaaatctccgcgcagtttgcaatcaccacaatcgccttctagtagttcaaagcgcaaatcacgcagaaacactgatgcaactcctcaaaagaagaaggcttaccgccgtaagccgggcactgtggcactctgggaaatacgcaaatttcagaagtcattcaagcccttgattcctgctgcgcctttcattcgaacagtgagagagattactcaccagtttgctccttatgttggtcgttggcaagctgaagctctgatggcccttcaagaggctgcagagaattttattgtccgtttgtttgaagatggtatgctttgtgcaattcatgccaaacgagttacactcatgaaaaaggatttggagctcgcgcgaaggattgggggcagagagaggggatggtaa

SEQ ID NO: 44 - protein, 154 aa, Beta vulgaris
MRVKHTAARKSTTNGPRSKAQKSPRSLQSPQSPSSSSKRKSRRNTDATPQKKKAYRRKPGTVALWEIRKFQKSFKPLIPAAPFIRTVREITHQFAPYVGRWQAEALMALQEAAENFIVRLFEDGMLCAIHAKRVTLMKKDLELARRIGGRERGW

SEQ ID NO: 45 - DNA, 465 bp, Beta vulgaris
atgagagttaaacacactgctgccaggaaatcaaccaccaatggtcctcgttcaaaggctcagaaatctccgcgcagtttgcaatcaccacaatcgccttctagtagttcaaagcgcaaatcacgcagaaacactgatgcaactcctcaaaagaagaaggcttaccgccgtaagccgggcactgtggcactctgggaaatacgcaaatttcagaagtcattcaagcccttgattcctgctgcgcctttcattcgaacagtgagagagattactcaccagtttgctccttatgttggtcgttggcaagctgaagcttttatggcccttcaagaggctgcagagaattttattgtccgtttgtttgaagatggtatgctttgtgcaattcatgccaaacgagttacactcatgaaaaaggatttggagctcgcgcgaaggattgggggcagagagaggggatggtaa

SEQ ID NO: 46 - protein, 154 aa, Beta vulgaris
MRVKHTAARKSTTNGPRSKAQKSPRSLQSPQSPSSSSKRKSRRNTDATPQKKKAYRRKPGTVALWEIRKFQKSFKPLIPAAPFIRTVREITHQFAPYVGRWQAEAFMALQEAAENFIVRLFEDGMLCAIHAKRVTLMKKDLELARRIGGRERGW

SEQ ID NO: 47 - DNA, 465 bp, Beta vulgaris
atgagagttaaacacactgctgccaggaaatcaaccaccaatggtcctcgttcaaaggctcagaaatctccgcgcagtttgcaatcaccacaatcgccttctagtagttcaaagcgcaaatcacgcagaaacactgatgcaactcctcaaaagaagaaggcttaccgccgtaagccgggcactgtggcactctgggaaatacgcaaatttcagaagtcattcaagcccttgattcctgctgcgcctttcattcgaacagtgagagagattactcaccagtttgctccttatgttggtcgttggcaagctgaagctattatggcccttcaagaggctgcagagaattttattgtccgtttgtttgaagatggtatgctttgtgcaattcatgccaaacgagttacactcatgaaaaaggatttggagctcgcgcgaaggattgggggcagagagaggggatggtaa

SEQ ID NO: 48 - protein, 154 aa, Beta vulgaris
MRVKHTAARKSTTNGPRSKAQKSPRSLQSPQSPSSSSKRKSRRNTDATPQKKKAYRRKPGTVALWEIRKFQKSFKPLIPAAPFIRTVREITHQFAPYVGRWQAEAIMALQEAAENFIVRLFEDGMLCAIHAKRVTLMKKDLELARRIGGRERGW